European Patent Application EP 4 321 170 A1, published February 14, 2024. Title: A composition comprising a glucagon derivative for preventing or treating chronic kidney disease. Applicant: HANMI PHARM. CO., LTD. The sequence listing filed with the application follows.

SEQUENCE LISTING (73 sequences)

SEQ ID NO: 1 - protein, 29 aa, homo sapiens
HSQGTFTSDYSKYLDSRRAQDFVQWLMNT

SEQ ID NO: 2 - protein, 29 aa, Artificial Sequence
  glucagon derivative
HSQGTFTSDYSKYLDCDRAQDFVQWLMNT

SEQ ID NO: 3 - protein, 29 aa, Artificial Sequence
  glucagon derivative
HSQGTFTSDYSKYLDCERAQDFVQWLMNT

SEQ ID NO: 4 - protein, 29 aa, Artificial Sequence
  glucagon derivative
HSQGTFTSDYSKYLDSCDAQDFVQWLMNT

SEQ ID NO: 5 - protein, 29 aa, Artificial Sequence
  glucagon derivative
HSQGTFTSDYSKYLDSCEAQDFVQWLMNT

SEQ ID NO: 6 - protein, 29 aa, Artificial Sequence
  glucagon derivative
HSQGTFTSDYSKYLDSCEADDFVQWLMNT

SEQ ID NO: 7 - protein, 29 aa, Artificial Sequence
  glucagon derivative
YSQGTFTSDYSKYLDSCEADDFVQWLMNT

SEQ ID NO: 8 - protein, 29 aa, Artificial Sequence
  glucagon derivative
  MISC_FEATURE (2): Xaa is aminoisobutyric acid (Aib)
YXQGTFTSDYSKYLDSCDAQDFVQWLINT

SEQ ID NO: 9 - protein, 29 aa, Artificial Sequence
  glucagon derivative
  MISC_FEATURE (2): Xaa is aminoisobutyric acid (Aib)
YXQGTFTSDYSKYLDSCDAQDFVVWLINT

SEQ ID NO: 10 - protein, 29 aa, Artificial Sequence
  glucagon derivative
  MISC_FEATURE (2): Xaa is aminoisobutyric acid (Aib)
YXQGTFTSDYSKYLDSCDADDFVVWLINT

SEQ ID NO: 11 - protein, 29 aa, Artificial Sequence
  glucagon derivative
  MISC_FEATURE (2): Xaa is aminoisobutyric acid (Aib)
YXQGTFTSDYSKYLDEKCAKEFVQWLMNT

SEQ ID NO: 12 - protein, 30 aa, Artificial Sequence
  glucagon derivative
  MISC_FEATURE (2): Xaa is aminoisobutyric acid (Aib)
  MISC_FEATURE (16)..(20): amino acids at positions 16 and 20 form a ring
YXQGTFTSDYSKYLDEKRAKEFVQWLMNTC

SEQ ID NO: 13 - protein, 29 aa, Artificial Sequence
  glucagon derivative
  MISC_FEATURE (2): Xaa is aminoisobutyric acid (Aib)
YXQGTFTSDYSCYLDSRRAQDFVQWLMNT

SEQ ID NO: 14 - protein, 29 aa, Artificial Sequence
  glucagon derivative
  MISC_FEATURE (2): Xaa is aminoisobutyric acid (Aib)
YXQGTFTSDYSKYLDCKRAKEFVQWLMNT

SEQ ID NO: 15 - protein, 29 aa, Artificial Sequence
  glucagon derivative
  MISC_FEATURE (2): Xaa is aminoisobutyric acid (Aib)
YXQGTFTSDYSKYLCEKRAQDFVVWLMNT

SEQ ID NO: 16 - protein, 29 aa, Artificial Sequence
  glucagon derivative
  MISC_FEATURE (2): Xaa is aminoisobutyric acid (Aib)
YXQGTFTSDYSKYLDCRRAQVFVQWLMRT

SEQ ID NO: 17 - protein, 29 aa, Artificial Sequence
  glucagon derivative
  MISC_FEATURE (2): Xaa is aminoisobutyric acid (Aib)
YXQGTFTSDYSKYLDCVRAQDFVQWLMRT

SEQ ID NO: 18 - protein, 29 aa, Artificial Sequence
  glucagon derivative
  MISC_FEATURE (2): Xaa is aminoisobutyric acid (Aib)
YXQGTFTSDYSKYLDSRRACDFRLWLMNT

SEQ ID NO: 19 - protein, 29 aa, Artificial Sequence
  glucagon derivative
  MISC_FEATURE (2): Xaa is aminoisobutyric acid (Aib)
  MISC_FEATURE (16)..(20): amino acids at positions 16 and 20 form a ring
YXQGTFTSDYSKYLCEKRAKEFVQWLMNT

SEQ ID NO: 20 - protein, 29 aa, Artificial Sequence
  glucagon derivative
  MISC_FEATURE (2): Xaa is aminoisobutyric acid (Aib)
  MISC_FEATURE (16)..(20): amino acids at positions 16 and 20 form a ring
YXQGTFTSDYSKYLDECRAKEFVQWLMNT

SEQ ID NO: 21 - protein, 29 aa, Artificial Sequence
  glucagon derivative
  MISC_FEATURE (2): Xaa is aminoisobutyric acid (Aib)
  MISC_FEATURE (16)..(20): amino acids at positions 16 and 20 form a ring
YXQGTFTSDYSKYLDEKCAKEFVQWLMNT

SEQ ID NO: 22 - protein, 29 aa, Artificial Sequence
  glucagon derivative
  MISC_FEATURE (2): Xaa is aminoisobutyric acid (Aib)
  MISC_FEATURE (16)..(20): amino acids at positions 16 and 20 form a ring
YXQGTFTSDYSKYLDEKRCKEFVQWLMNT

SEQ ID NO: 23 - protein, 29 aa, Artificial Sequence
  glucagon derivative
  MISC_FEATURE (2): Xaa is aminoisobutyric acid (Aib)
  MISC_FEATURE (16)..(20): amino acids at positions 16 and 20 form a ring
YXQGTFTSDYSKYCDEKRAKEFVQWLMNT

SEQ ID NO: 24 - protein, 29 aa, Artificial Sequence
  glucagon derivative
  MISC_FEATURE (2): Xaa is aminoisobutyric acid (Aib)
  MISC_FEATURE (16)..(20): amino acids at positions 16 and 20 form a ring
YXQGTFTSDYSKCLDEKRAKEFVQWLMNT

SEQ ID NO: 25 - protein, 29 aa, Artificial Sequence
  glucagon derivative
  MISC_FEATURE (2): Xaa is aminoisobutyric acid (Aib)
  MISC_FEATURE (16)..(20): amino acids at positions 16 and 20 form a ring
YXQGTFTSDYSKYLDEKRAKCFVQWLMNT

SEQ ID NO: 26 - protein, 29 aa, Artificial Sequence
  glucagon derivative
  MISC_FEATURE (2): Xaa is aminoisobutyric acid (Aib)
  MISC_FEATURE (16)..(20): amino acids at positions 16 and 20 form a ring
WXQGTFTSDYSKYLDECRAKDFVQWLMNT

SEQ ID NO: 27 - protein, 29 aa, Artificial Sequence
  glucagon derivative
  MISC_FEATURE (2): Xaa is aminoisobutyric acid (Aib)
  MISC_FEATURE (16)..(20): amino acids at positions 16 and 20 form a ring
YXQGTFVSDYSKYLDECRAKDFVQWLMNT

SEQ ID NO: 28 - protein, 29 aa, Artificial Sequence
  glucagon derivative
  MISC_FEATURE (2): Xaa is aminoisobutyric acid (Aib)
  MISC_FEATURE (16)..(20): amino acids at positions 16 and 20 form a ring
WXQGTFVSDYSKYLDECRAKDFVQWLMNT

SEQ ID NO: 29 - protein, 29 aa, Artificial Sequence
  glucagon derivative
  MISC_FEATURE (2): Xaa is aminoisobutyric acid (Aib)
  MISC_FEATURE (16)..(20): amino acids at positions 16 and 20 form a ring
YXQGTFTSDYSKCLDERRAKDFVQWLMNT

SEQ ID NO: 30 - protein, 29 aa, Artificial Sequence
  glucagon derivative
  MISC_FEATURE (2): Xaa is aminoisobutyric acid (Aib)
  MISC_FEATURE (16)..(20): amino acids at positions 16 and 20 form a ring
WXQGTFTSDYSKCLDERRAKDFVQWLMNT

SEQ ID NO: 31 - protein, 29 aa, Artificial Sequence
  glucagon derivative
  MISC_FEATURE (2): Xaa is aminoisobutyric acid (Aib)
  MISC_FEATURE (17)..(21): amino acids at positions 17 and 21 form a ring
YXQGTFTSDYSKYLDCKRAKEFVQWLMNT

SEQ ID NO: 32 - protein, 28 aa, Artificial Sequence
  glucagon derivative
  MISC_FEATURE (15)..(19): amino acids at positions 15 and 19 form a ring
SQGTFTSDYSKYLDECRAKEFVQWLMNT

SEQ ID NO: 33 - protein, 29 aa, Artificial Sequence
  glucagon derivative
  MISC_FEATURE (2): Xaa is aminoisobutyric acid (Aib)
YXQGTFTSDYSKYLDSRRAQDFVQWLMNT

SEQ ID NO: 34 - protein, 29 aa, Artificial Sequence
  glucagon derivative
  MISC_FEATURE (2): Xaa is aminoisobutyric acid (Aib)
  MISC_FEATURE (16)..(20): amino acids at positions 16 and 20 form a ring
WXQGTFTSDYSKYCDERRAKEFVQWLMNT

SEQ ID NO: 35 - protein, 29 aa, Artificial Sequence
  glucagon derivative
  MISC_FEATURE (2): Xaa is aminoisobutyric acid (Aib)
  MISC_FEATURE (16)..(20): amino acids at positions 16 and 20 form a ring
YXQGTFTSDYSKYCDERRAKEFVQWLMNT

SEQ ID NO: 36 - protein, 29 aa, Artificial Sequence
  glucagon derivative
  MISC_FEATURE (2): Xaa is aminoisobutyric acid (Aib)
  MISC_FEATURE (16)..(20): amino acids at positions 16 and 20 form a ring
YXQGTFTSDCSKYLDERRAKEFVQWLMNT

SEQ ID NO: 37 - protein, 30 aa, Artificial Sequence
  glucagon derivative
  MISC_FEATURE (2): Xaa is aminoisobutyric acid (Aib)
  MISC_FEATURE (16)..(20): amino acids at positions 16 and 20 form a ring
YXQGTFTSDYSKYLDERRAKEFVQWLMNTC

SEQ ID NO: 38 - protein, 29 aa, Artificial Sequence
  glucagon derivative
  MISC_FEATURE (2): Xaa is aminoisobutyric acid (Aib)
  MISC_FEATURE (16)..(20): amino acids at positions 16 and 20 form a ring
YXQGTFCSDYSKYLDERRAKEFVQWLMNT

SEQ ID NO: 39 - protein, 29 aa, Artificial Sequence
  glucagon derivative
  MISC_FEATURE (2): Xaa is aminoisobutyric acid (Aib)
  MISC_FEATURE (16)..(20): amino acids at positions 16 and 20 form a ring
YXQGTFVSDCSKYLDERRAKDFVQWLMNT

SEQ ID NO: 40 - protein, 30 aa, Artificial Sequence
  glucagon derivative
  MISC_FEATURE (2): Xaa is aminoisobutyric acid (Aib)
  MISC_FEATURE (16)..(20): amino acids at positions 16 and 20 form a ring
YXQGTFVSDYSKYLDERRAKDFVQWLMNTC

SEQ ID NO: 41 - protein, 29 aa, Artificial Sequence
  glucagon derivative
  MISC_FEATURE (2): Xaa is aminoisobutyric acid (Aib)
  MISC_FEATURE (16)..(20): amino acids at positions 16 and 20 form a ring
YXQGTFCSDYSKYLDERRAKDFVQWLMNT

SEQ ID NO: 42 - protein, 29 aa, Artificial Sequence
  glucagon derivative
  MISC_FEATURE (2): Xaa is aminoisobutyric acid (Aib)
YXQGTFCSDYSKYLDSRRAQDFVQWLMNT

SEQ ID NO: 43 - protein, 29 aa, Artificial Sequence
  glucagon derivative
  MISC_FEATURE (2): Xaa is aminoisobutyric acid (Aib)
YXQGTFTSDCSKYLDSRRAQDFVQWLMNT

SEQ ID NO: 44 - protein, 30 aa, Artificial Sequence
  glucagon derivative
  MISC_FEATURE (2): Xaa is aminoisobutyric acid (Aib)
YXQGTFTSDYSKYLDSRRAQDFVQWLMNTC

SEQ ID NO: 45 - protein, 29 aa, Artificial Sequence
  glucagon derivative
  MISC_FEATURE (2): Xaa is aminoisobutyric acid (Aib)
YXQGTFTSDYSCYLDEKRAKEFVQWLMNT

SEQ ID NO: 46 - protein, 30 aa, Artificial Sequence
  General Formula 1
  MISC_FEATURE (1): Xaa is tyrosine
  MISC_FEATURE (2): Xaa is alpha-methyl-glutamic acid, aminoisobutyric acid (Aib), D-alanine, glycine, Sar (N-methylglycine), serine, or D-serine
  MISC_FEATURE (7): Xaa is threonine, valine, or cysteine
  MISC_FEATURE (10): Xaa is tyrosine or cysteine
  MISC_FEATURE (12): Xaa is lysine or cysteine
  MISC_FEATURE (13): Xaa is tyrosine or cysteine
  MISC_FEATURE (14): Xaa is leucine or cysteine
  MISC_FEATURE (15): Xaa is aspartic acid, glutamic acid, or cysteine
  MISC_FEATURE (16): Xaa is glutamic acid, aspartic acid, serine, alpha-methyl-glutamic acid, or cysteine, or is absent;
  MISC_FEATURE (17): Xaa is aspartic acid, glutamine, glutamic acid, lysine, arginine, serine, cysteine, or valine, or is absent
  MISC_FEATURE (18): Xaa is alanine, aspartic acid, glutamic acid, arginine, valine, or cysteine, or is absent
  MISC_FEATURE (19): Xaa is alanine, arginine, serine, valine, or cysteine, or is absent
  MISC_FEATURE (20): Xaa is lysine, histidine, glutamine, aspartic acid, arginine, alpha-methyl-glutamic acid, or cysteine, or is absent
  MISC_FEATURE (21): Xaa is aspartic acid, glutamic acid, leucine, valine, or cysteine, or is absent
  MISC_FEATURE (23): Xaa is isoleucine, valine, or arginine, or is absent
  MISC_FEATURE (24): Xaa is valine, arginine, alanine, cysteine, glutamic acid, lysine, glutamine, alpha-methyl-glutamic acid, or leucine, or is absent;
  MISC_FEATURE (27): Xaa is isoleucine, valine, alanine, lysine, methionine, glutamine, or arginine, or is absent
  MISC_FEATURE (28): Xaa is glutamine, lysine, asparagine, or arginine, or is absent
  MISC_FEATURE (29): Xaa is threonine
  MISC_FEATURE (30): Xaa is cysteine, or is absent
XXQGTFXSDXSXXXXXXXXXXFXXWLXXXX

SEQ ID NO: 47 - protein, 12 aa, homo sapiens
ESKYGPPCPSCP

SEQ ID NO: 48 - protein, 11 aa, Artificial Sequence
  Variant of hinge region
ESKYGPPPSCP

SEQ ID NO: 49 - protein, 11 aa, Artificial Sequence
  Variant of hinge region
ESKYGPPCPSP

SEQ ID NO: 50 - protein, 10 aa, Artificial Sequence
  Variant of hinge region
ESKYGPPCPS

SEQ ID NO: 51 - protein, 10 aa, Artificial Sequence
  Variant of hinge region
ESKYGPPCPP

SEQ ID NO: 52 - protein, 8 aa, Artificial Sequence
  Variant of hinge region
KYGPPCPS

SEQ ID NO: 53 - protein, 8 aa, Artificial Sequence
  Variant of hinge region
ESKYGPPC

SEQ ID NO: 54 - protein, 7 aa, Artificial Sequence
  Variant of hinge region
EKYGPPC

SEQ ID NO: 55 - protein, 6 aa, Artificial Sequence
  Variant of hinge region
ESPSCP

SEQ ID NO: 56 - protein, 5 aa, Artificial Sequence
  Variant of hinge region
EPSCP

SEQ ID NO: 57 - protein, 4 aa, Artificial Sequence
  Variant of hinge region
PSCP

SEQ ID NO: 58 - protein, 10 aa, Artificial Sequence
  Variant of hinge region
ESKYGPPSCP

SEQ ID NO: 59 - protein, 9 aa, Artificial Sequence
  Variant of hinge region
KYGPPPSCP

SEQ ID NO: 60 - protein, 9 aa, Artificial Sequence
  Variant of hinge region
ESKYGPSCP

SEQ ID NO: 61 - protein, 8 aa, Artificial Sequence
  Variant of hinge region
ESKYGPPC

SEQ ID NO: 62 - protein, 7 aa, Artificial Sequence
  Variant of hinge region
KYGPPCP

SEQ ID NO: 63 - protein, 7 aa, Artificial Sequence
  Variant of hinge region
ESKPSCP

SEQ ID NO: 64 - protein, 6 aa, Artificial Sequence
  Variant of hinge region
ESPSCP

SEQ ID NO: 65 - protein, 4 aa, Artificial Sequence
  Variant of hinge region
EPSC

SEQ ID NO: 66 - protein, 3 aa, Artificial Sequence
  Variant of hinge region
SCP

SEQ ID NO: 67 - protein, 221 aa, homo sapiens
PSCPAPEFLGGPSVFLFPPKPKDTLMISRTPEVTCVVVDVSQEDPEVQFNWYVDGVEVHNAKTKPREEQFNSTYRVVSVLTVLHQDWLNGKEYKCKVSNKGLPSSIEKTISKAKGQPREPQVYTLPPSQEEMTKNQVSLTCLVKGFYPSDIAVEWESNGQPENNYKTTPPVLDSDGSFFLYSRLTVDKSRWQEGNVFSCSVMHEALHNHYTQKSLSLSLGK

SEQ ID NO: 68 - protein, 442 aa, Homo sapiens
  MISC_FEATURE (1)..(442): Amino acids at position 1 to 442 form Human Immunoglobulin G4 Fc Fragment (homodimer)
  MISC_FEATURE (1)..(221): Amino acids at position 1 to 221 form one monomer
  MISC_FEATURE (222)..(442): Amino acids at position 222 to 442 form one monomer
  DISULFID (3)..(224): Amino acids at position 3 and position 224 form an inter-disulfide bond
  DISULFID (35)..(95): Amino acids at position 35 and position 95 form an intra-chain disulfide bond
  DISULFID (141)..(199): Amino acids at position 141 and position 199 form an intra-chain disulfide bond
  DISULFID (256)..(316): Amino acids at position 256 and position 316 form an intra-chain disulfide bond
  DISULFID (362)..(420): Amino acids at position 362 and position 420 form an intra-chain disulfide bond
PSCPAPEFLGGPSVFLFPPKPKDTLMISRTPEVTCVVVDVSQEDPEVQFNWYVDGVEVHNAKTKPREEQFNSTYRVVSVLTVLHQDWLNGKEYKCKVSNKGLPSSIEKTISKAKGQPREPQVYTLPPSQEEMTKNQVSLTCLVKGFYPSDIAVEWESNGQPENNYKTTPPVLDSDGSFFLYSRLTVDKSRWQEGNVFSCSVMHEALHNHYTQKSLSLSLGKPSCPAPEFLGGPSVFLFPPKPKDTLMISRTPEVTCVVVDVSQEDPEVQFNWYVDGVEVHNAKTKPREEQFNSTYRVVSVLTVLHQDWLNGKEYKCKVSNKGLPSSIEKTISKAKGQPREPQVYTLPPSQEEMTKNQVSLTCLVKGFYPSDIAVEWESNGQPENNYKTTPPVLDSDGSFFLYSRLTVDKSRWQEGNVFSCSVMHEALHNHYTQKSLSLSLGK

SEQ ID NO: 69 - protein, 31 aa, homo sapiens
HAEGTFTSDVSSYLEGQAAKEFIAWLVKGRG

SEQ ID NO: 70 - protein, 39 aa, Artificial Sequence
  Exendin-3
HSDGTFTSDLSKQMEEEAVRLFIEWLKNGGPSSGAPPPS

SEQ ID NO: 71 - protein, 39 aa, Artificial Sequence
  Exendin-4
HGEGTFTSDLSKQMEEEAVRLFIEWLKNGGPSSGAPPPS

SEQ ID NO: 72 - protein, 38 aa, Artificial Sequence
  GLP-1 receptor agonist
  MISC_FEATURE (1): 1H-imidazol-4-yl-acetyl is linked to the amino group of Gly
GEGTFTSDLSKQMEEEAVRLFIEWLKNGGPSSGAPPPS

SEQ ID NO: 73 - protein, 29 aa, Artificial Sequence
  GLP-1 receptor agonist
HGEGTFTSDVSSYLEEQAAKEFIAWLVKG